European Patent Specification EP 3 539 992 B1, published December 13, 2023. Title: Fragment antibody and method for protein crystallization using fragment antibody. Applicant: Wako Pure Chemical lndustries ltd. The sequence listing filed with the application follows.

SEQUENCE LISTING (89 sequences)

SEQ ID NO: 1 - protein, 49 aa, Homo sapiens
DYEFLKSWTVEDLQKRLLALDPMMWQEIEEIRQKYQSKRQPILDAIEAK

SEQ ID NO: 2 - protein, 49 aa, Homo sapiens
DFDFLKNLSLEELQMRLKALDPMMEREIEELRQRYTAQRQPILDAMDAK

SEQ ID NO: 3 - protein, 48 aa, Drosophila
FEFLKFLTFDDLNQRLCNIDHEMELEIEQLNKKYNAKRQPIVDAMNAK

SEQ ID NO: 4 - protein, 47 aa, Drosophila
VAQFLNLSLPECRAILERYDELAREVAKIKERYAELRRRIVSRMESL

SEQ ID NO: 5 - protein, 48 aa, Homo sapiens
EVEWDAFSIPELQNFLTILEKEEQDKIQQVQKKYDKFRQKLEEALRES

SEQ ID NO: 6 - protein, 48 aa, Homo sapiens
EVNWDAFSMPELHNFLRILQREEEEHLRQILQKYSYCRQKIQEALHAC

SEQ ID NO: 7 - protein, 48 aa, Homo sapiens
ILKWELFQLADLDTYQGMLKLLFMKELEQIVKLYEAYRQALLTELENR

SEQ ID NO: 8 - protein, 48 aa, Drosophila
LLQFNMFSLPELEGFDSMLVRLFKQELGTIVGFYERYRRALILEKNRR

SEQ ID NO: 9 - protein, 49 aa, Artificial Sequence
  Mutated Mst1 SARAH Domain
DYEFLKSWTVEDLQKRLLALDPMMWQEIEEIRQKYQCKRQPILDAIEAK

SEQ ID NO: 10 - protein, 49 aa, Artificial Sequence
  Mutated Mst2 SARAH Domain
DFDFLKNLSLEELQMRLKALDPMMEREIEELRQRYTCQRQPILDAMDAK

SEQ ID NO: 11 - protein, 48 aa, Artificial Sequence
  Mutated Hippo SARAH Domain
FEFLKFLTFDDLNQRLCNIDHEMELEIEQLNKKYNCKRQPIVDAMNAK

SEQ ID NO: 12 - protein, 47 aa, Artificial Sequence
  Mutated RASSF SARAH Domain
VAQFLNLSLPECRAILERYDELAREVAKIKERYACLRRRIVSRMESL

SEQ ID NO: 13 - protein, 48 aa, Artificial Sequence
  Mutated RASSF5 SARAH Domain
EVEWDAFSIPELQNFLTILEKEEQDKIQQVQKKYDCFRQKLEEALRES

SEQ ID NO: 14 - protein, 48 aa, Artificial Sequence
  Mutated RASSF1 SARAH Domain
EVNWDAFSMPELHNFLRILQREEEEHLRQILQKYSCCRQKIQEALHAC

SEQ ID NO: 15 - protein, 48 aa, Artificial Sequence
  Mutated WW45 SARAH Domain
ILKWELFQLADLDTYQGMLKLLFMKELEQIVKLYECYRQALLTELENR

SEQ ID NO: 16 - protein, 48 aa, Artificial Sequence
  Mutated Sav SARAH Domain
LLQFNMFSLPELEGFDSMLVRLFKQELGTIVGFYECYRRALILEKNRR

SEQ ID NO: 17 - protein, 168 aa, Artificial Sequence
  VH-SARAH(Y35C) of P20.1 Antibody
MQIQLVQSGPEVQKPGETVRISCKASGYTFTTAGMQWVQKMPGKSLKWIGWINTRSGVPKYAEDFKGRFAFSLETSASIAYLHINNLKNEDTATYFCAREGPGFVYWGQGTLVTVSSGSDYEFLKSWTVEDLQKRLLALDPMMEQEIEEIRQKCQSKRQPILDAIEAK

SEQ ID NO: 18 - protein, 163 aa, Artificial Sequence
  VL-SARAH(M24C) of P20.1 Antibody
MGQTVVTQESALTTSPGETVTLTCRSSTGAVTTSNYANWVQEKPDHLFTGLIVGTNNRVPGVPPRFSGSLIEDKAALTITGAQTEDEAIYFCALWYSNHWVFGGGTKLTVLGGSDYEFLKSWTVEDLQKRLLALDPMCEQEIEEIRQKYQSKRQPILDAIEAK

SEQ ID NO: 19 - DNA, 507 bp, Artificial Sequence
  VH-SARAH(Y35C) of P20.1 Antibody
atgcagatccagttggtgcagtctggacctgaggtgcagaagcctggagagacagtcaggatctcctgcaaggcttctgggtataccttcacaactgctggaatgcagtgggtgcaaaagatgccaggaaagagtttgaagtggattggctggataaacacccgctctggagtgccaaaatatgcagaagacttcaagggacgttttgccttctctttggaaacctctgccagtattgcatatttacatataaacaacctcaaaaatgaggacacggctacctatttctgtgcgagagaggggcctggatttgtttactggggccaagggactctggtcaccgtctcgagcggatccgactacgagtttcttaagagttggacagtggaggaccttcagaagaggctcttggccctggaccccatgatggagcaggagattgaagagatccggcagaagtgccagtccaagcggcagcccatcctggatgccatagaggctaagtag

SEQ ID NO: 20 - DNA, 510 bp, Artificial Sequence
  VL-SARAH(M24C) of P20.1 Antibody
atgggccagatccagttggtgcagtctggacctgaggtgcagaagcctggagagacagtcaggatctcctgcaaggcttctgggtataccttcacaactgctggaatgcagtgggtgcaaaagatgccaggaaagagtttgaagtggattggctggataaacacccgctctggagtgccaaaatatgcagaagacttcaagggacgttttgccttctctttggaaacctctgccagtattgcatatttacatataaacaacctcaaaaatgaggacacggctacctatttctgtgcgagagaggggcctggatttgtttactggggccaagggactctggtcaccgtctcgagcggatccgactacgagtttcttaagagttggacagtggaggaccttcagaagaggctcttggccctggaccccatgatggagcaggagattgaagagatccggcagaagtgccagtccaagcggcagcccatcctggatgccatagaggctaagtag

SEQ ID NO: 21 - protein, 8 aa, Artificial Sequence
  C8 Peptide
PRGYPGQV

SEQ ID NO: 22 - protein, 196 aa, Artificial Sequence
  VH-SARAH(Y35C) of P20.1 Antibody
MLDASGCSWMWTWALLQLLLLVGPGGCGRQIQLVQSGPEVQKPGETVRISCKASGYTFTTAGMQWVQKMPGKSLKWIGWINTRSGVPKYAEDFKGRFAFSLETSASIAYLHINNLKNEDTATYFCAREGPGFVYWGQGTLVTVSSGSDYEFLKSWTVEDLQKRLLALDPMMEQEIEEIRQKCQSKRQPILDAIEAK

SEQ ID NO: 23 - DNA, 594 bp, Artificial Sequence
  VH-SARAH(Y35C) of P20.1 Antibody
atgctggacgcgagcggctgtagttgggcgatgtggacgtgggcgctgttgcagctgctgctactagtggggcccggaggctgcggccgccagatccagttggtgcagtctggacctgaggtgcagaagcctggagagacagtcaggatctcctgcaaggcttctgggtataccttcacaactgctggaatgcagtgggtgcaaaagatgccaggaaagagtttgaagtggattggctggataaacacccgctctggagtgccaaaatatgcagaagacttcaagggacgttttgccttctctttggaaacctctgccagtattgcatatttacatataaacaacctcaaaaatgaggacacggctacctatttctgtgcgagagaggggcctggatttgtttactggggccaagggactctggtcaccgtctcgagcggatccgactacgagtttcttaagagttggacagtggaggaccttcagaagaggctcttggccctggaccccatgatggagcaggagattgaagagatccggcagaagtgccagtccaagcggcagcccatcctggatgccatagaggctaagtaa

SEQ ID NO: 24 - protein, 191 aa, Artificial Sequence
  VL-SARAH(M24C) of P20.1 Antibody
MLDASGCSWMWTWALLQLLLLVGPGGCGRTQTVVTQESALTTSPGETVTLTCRSSTGAVTTSNYANWVQEKPDHLFTGLIVGTNNRVPGVPPRFSGSLIEDKAALTITGAQTEDEAIYFCALWYSNHWVFGGGTKLTVLGGSDYEFLKSWTVEDLQKRLLALDPMCEQEIEEIRQKYQSKRQPILDAIEAK

SEQ ID NO: 25 - DNA, 579 bp, Artificial Sequence
  VL-SARAH(M24C) of P20.1 Antibody
atgctggacgcgagcggctgtagttgggcgatgtggacgtgggcgctgttgcagctgctgctactagtggggcccggaggctgcggccgcacgcagactgttgtgactcaggaatctgctctcaccacatcacctggtgaaacagtcacactcacttgtcgctcaagtactggggctgttacaactagtaactatgccaactgggtccaagaaaaaccagatcatttattcactggtctaatagttggtaccaacaaccgagttccaggtgttcctcccagattctcaggctccctgattgaagacaaggctgccctcaccatcacaggggcacagactgaggatgaggcaatatatttctgtgctctatggtacagcaaccattgggtgttcggtggaggaaccaaactgactgtcctaggcggatccgactacgagtttcttaagagttggacagtggaggaccttcagaagaggctcttggccctggaccccatgtgcgagcaggagattgaagagatccggcagaagtaccagtccaagcggcagcccatcctggatgccatagaggctaagtaa

SEQ ID NO: 26 - DNA, 519 bp, Artificial Sequence
  VH-SARAH(Y35C) of 12CA5 Antibody
atggaagtgaagttggttgaatctgggggagacctggtgaaaccgggcgggagtctgaaactgtcctgtgcggcaagtggctttaccttctcatcctacggcatgtcctgggttcgtcagaccccggataagcgtctggaatgggtcgcaactatttctcggggcggtagttatacctattaccccgattcagtgaaaggccggtttacaatcagccgcgacaacgctaagaatactctgtacctgcagatgagctccctgaaatctgaggataccgccatgtattactgcgcgcgccgtgaaacctatgatgagaaaggtttcgcctactgggggcagggaaccacagtgaccgtttcctcaggatccgactacgagtttcttaagagttggacagtggaggaccttcagaagaggctcttggccctggaccccatgatggagcaggagattgaagagatccggcagaagtgccagtccaagcggcagcccatcctggatgccatagaggctaagtag

SEQ ID NO: 27 - DNA, 501 bp, Artificial Sequence
  VL-SARAH(M24C) of 12CA5 Antibody
atggacatcgaattgactcagtctccgtctagcctgaccgttactgcgggagagaaagttacaatgagctgtaagtcttcccagagcctgctgaatagcggcaaccagaaaaactatctgacctggtaccagcagaaacctggtcagccgcccaagctgctgatctattgggcatcaacacgcgaaagcggcgtgcctgatcgttttaccggctctggtagtgggcgggacttcaccctgacaatcagctccgtgcaggccgaagatctggcggtttattactgccagaacgacaattctcacccgctgacttttggagccggcaccaaactggagctgaaagcgggatccgactacgagtttcttaagagttggacagtggaggaccttcagaagaggctcttggccctggaccccatgtgcgagcaggagattgaagagatccggcagaagtaccagtccaagcggcagcccatcctggatgccatagaggctaagtag

SEQ ID NO: 28 - protein, 172 aa, Artificial Sequence
  VH-SARAH(Y35C) of 12CA5 Antibody
MEVKLVESGGDLVKPGGSLKLSCAASGFTFSSYGMSWVRQTPDKRLEWVATISRGGSYTYYPDSVKGRFTISRDNAKNTLYLQMSSLKSEDTAMYYCARRETYDEKGFAYWGQGTTVTVSSGSDYEFLKSWTVEDLQKRLLALDPMMEQEIEEIRQKCQSKRQPILDAIEAK

SEQ ID NO: 29 - protein, 166 aa, Artificial Sequence
  VL-SARAH(M24C) of 12CA5 Antibody
MDIELTQSPSSLTVTAGEKVTMSCKSSQSLLNSGNQKNYLTWYQQKPGQPPKLLIYWASTRESGVPDRFTGSGSGRDFTLTISSVQAEDLAVYYCQNDNSHPLTFGAGTKLELKAGSDYEFLKSWTVEDLQKRLLALDPMCEQEIEEIRQKYQSKRQPILDAIEAK

SEQ ID NO: 30 - protein, 9 aa, Artificial Sequence
  HA peptide
YPYDVPDYA

SEQ ID NO: 31 - protein, 193 aa, Artificial Sequence
  VH-SARAH of 2H5 Antibody
MLVLQWVLVTALFQGVHCAVQLVESGGGLVQPKESLKISCAAFGVTFSNVAMYWVRQAPGKGLEWIARIRTKPNNYATYYADSVKGRFTISRDDSKSMVYLQMDNLKTEDTAMYYCTAEVATDWGQGVMVTVSSRSDYEFLKSWTVEDLQKRLLALDPMMEQEIEEIRQKYQSKRQPILDAIEAKTGHHHHHH

SEQ ID NO: 32 - protein, 192 aa, Artificial Sequence
  VL-SARAH of 2H5 Antibody
MMSPVQSLFLLLLWILGTNGDVVLTQAPPTLSATIGQSVSISCRSSQSLLHRNGNTYLNWLLQRPGQPPQLLIYLVSRLESGVPNRFSGSGSGTAFTLKISGLEAEDLGVYYCVQGTHAPLTFGSGTKLEIKRGSDYEFLKSWTVEDLQKRLLALDPMMEQEIEEIRQKYQSKRQPILDAIEAKTGHHHHHH

SEQ ID NO: 33 - DNA, 582 bp, Artificial Sequence
  VH-SARAH of 2H5 Antibody
atgttggtgctgcagtgggttttggtgactgctctttttcaaggtgtgcattgtgcggtgcagcttgttgagtctggtggaggattggtgcagcctaaggagtcattgaaaatctcatgtgcagcctttggagtcaccttcagtaatgttgccatgtactgggtccgccaggctccaggaaagggtctggaatggattgctcgcataagaactaaacctaataattatgcaacatattatgctgattcagtgaaaggcagattcaccatctccagagatgattcaaaaagcatggtctacctacaaatggataacttgaaaactgaggacacagccatgtattactgtacagcagaagttgcaactgactggggccaaggagtcatggtcacagtctcctcaagatccgactacgagtttcttaagagttggacagtggaggaccttcagaagaggctcttggccctggaccccatgatggagcaggagattgaagagatccggcagaagtaccagtccaagcggcagcccatcctggatgccatagaggctaagaccggtcatcatcaccatcaccattga

SEQ ID NO: 34 - DNA, 579 bp, Artificial Sequence
  VL-SARAH of 2H5 Antibody
atgatgagtcctgtccagtccctgtttttgctattgctttggattctgggaaccaatggtgatgttgtgctgacccaggctccacccactttatcggctaccattggacaatcagtctccatctcttgcaggtcaagtcagagtctcttacatcgtaatggaaacacctatttaaattggttgctacagaggccaggccaacctccacaacttctaatttatttggtatccagactggaatctggggtccccaacaggttcagtggcagtgggtcaggaactgctttcacactcaaaatcagtggactagaggctgaggatttgggagtttattactgcgtgcaaggtacccatgctccgctcacgttcggttctgggaccaagctggagatcaaacggggatccgactacgagtttcttaagagttggacagtggaggaccttcagaagaggctcttggccctggaccccatgatggagcaggagattgaagagatccggcagaagtaccagtccaagcggcagcccatcctggatgccatagaggctaagaccggtcatcatcaccatcaccattga

SEQ ID NO: 35 - protein, 193 aa, Artificial Sequence
  VH(11C)-SARAH of 2H5 Antibody
MLVLQWVLVTALFQGVHCAVQLVESGGGCVQPKESLKISCAAFGVTFSNVAMYWVRQAPGKGLEWIARIRTKPNNYATYYADSVKGRFTISRDDSKSMVYLQMDNLKTEDTAMYYCTAEVATDWGQGVMVTVSSRSDYEFLKSWTVEDLQKRLLALDPMMEQEIEEIRQKYQSKRQPILDAIEAKTGHHHHHH

SEQ ID NO: 36 - protein, 192 aa, Artificial Sequence
  VL-SARAH(33C) of 2H5 Antibody
MMSPVQSLFLLLLWILGTNGDVVLTQAPPTLSATIGQSVSISCRSSQSLLHRNGNTYLNWLLQRPGQPPQLLIYLVSRLESGVPNRFSGSGSGTAFTLKISGLEAEDLGVYYCVQGTHAPLTFGSGTKLEIKRGSDYEFLKSWTVEDLQKRLLALDPMMEQEIECIRQKYQSKRQPILDAIEAKTGHHHHHH

SEQ ID NO: 37 - protein, 193 aa, Artificial Sequence
  VH(108C)-SARAH of 2H5 Antibody
MLVLQWVLVTALFQGVHCAVQLVESGGGLVQPKESLKISCAAFGVTFSNVAMYWVRQAPGKGLEWIARIRTKPNNYATYYADSVKGRFTISRDDSKSMVYLQMDNLKTEDTAMYYCTAEVATDWGQGVCVTVSSRSDYEFLKSWTVEDLQKRLLALDPMMEQEIEEIRQKYQSKRQPILDAIEAKTGHHHHHH

SEQ ID NO: 38 - protein, 192 aa, Artificial Sequence
  VL-SARAH(30C) of 2H5 Antibody
MMSPVQSLFLLLLWILGTNGDVVLTQAPPTLSATIGQSVSISCRSSQSLLHRNGNTYLNWLLQRPGQPPQLLIYLVSRLESGVPNRFSGSGSGTAFTLKISGLEAEDLGVYYCVQGTHAPLTFGSGTKLEIKRGSDYEFLKSWTVEDLQKRLLALDPMMEQEIEEIRCKYQSKRQPILDAIEAKTGHHHHHH

SEQ ID NO: 39 - protein, 193 aa, Artificial Sequence
  VH(112C)-SARAH of 2H5 Antibody
MLVLQWVLVTALFQGVHCAVQLVESGGGLVQPKESLKISCAAFGVTFSNVAMYWVRQAPGKGLEWIARIRTKPNNYATYYADSVKGRFTISRDDSKSMVYLQMDNLKTEDTAMYYCTAEVATDWGQGVMVTVCSRSDYEFLKSWTVEDLQKRLLALDPMMEQEIEEIRQKYQSKRQPILDAIEAKTGHHHHHH

SEQ ID NO: 40 - protein, 192 aa, Artificial Sequence
  VL-SARAH(37C) of 2H5 Antibody
MMSPVQSLFLLLLWILGTNGDVVLTQAPPTLSATIGQSVSISCRSSQSLLHRNGNTYLNWLLQRPGQPPQLLIYLVSRLESGVPNRFSGSGSGTAFTLKISGLEAEDLGVYYCVQGTHAPLTFGSGTKLEIKRGSDYEFLKSWTVEDLQKRLLALDPMMEQEIEEIRQKYQCKRQPILDAIEAKTGHHHHHH

SEQ ID NO: 41 - DNA, 507 bp, Artificial Sequence
  VH(112C)-SARAH of P20.1 Antibody
atgcagatccagttggtgcagtctggacctgaggtgcagaagcctggagagacagtcaggatctcctgcaaggcttctgggtataccttcacaactgctggaatgcagtgggtgcaaaagatgccaggaaagagtttgaagtggattggctggataaacacccgctctggagtgccaaaatatgcagaagacttcaagggacgttttgccttctctttggaaacctctgccagtattgcatatttacatataaacaacctcaaaaatgaggacacggctacctatttctgtgcgagagaggggcctggatttgtttactggggccaagggactctggtcaccgtctgcagcggatccgactacgagtttcttaagagttggacagtggaggaccttcagaagaggctcttggccctggaccccatgatggagcaggagattgaagagatccggcagaagtaccagtccaagcggcagcccatcctggatgccatagaggctaagtag

SEQ ID NO: 42 - DNA, 510 bp, Artificial Sequence
  VL-SARAH(37C) of P20.1 Antibody
atgggccagatccagttggtgcagtctggacctgaggtgcagaagcctggagagacagtcaggatctcctgcaaggcttctgggtataccttcacaactgctggaatgcagtgggtgcaaaagatgccaggaaagagtttgaagtggattggctggataaacacccgctctggagtgccaaaatatgcagaagacttcaagggacgttttgccttctctttggaaacctctgccagtattgcatatttacatataaacaacctcaaaaatgaggacacggctacctatttctgtgcgagagaggggcctggatttgtttactggggccaagggactctggtcaccgtctcgagcggatccgactacgagtttcttaagagttggacagtggaggaccttcagaagaggctcttggccctggaccccatgatggagcaggagattgaagagatccggcagaagtaccagtgcaagcggcagcccatcctggatgccatagaggctaagtag

SEQ ID NO: 43 - protein, 168 aa, Artificial Sequence
  VH(112C)-SARAH of P20.1 Antibody
MQIQLVQSGPEVQKPGETVRISCKASGYTFTTAGMQWVQKMPGKSLKWIGWINTRSGVPKYAEDFKGRFAFSLETSASIAYLHINNLKNEDTATYFCAREGPGFVYWGQGTLVTVCSGSDYEFLKSWTVEDLQKRLLALDPMMEQEIEEIRQKYQSKRQPILDAIEAK

SEQ ID NO: 44 - protein, 163 aa, Artificial Sequence
  VL-SARAH(37C) of P20.1 Antibody
MGQTVVTQESALTTSPGETVTLTCRSSTGAVTTSNYANWVQEKPDHLFTGLIVGTNNRVPGVPPRFSGSLIEDKAALTITGAQTEDEAIYFCALWYSNHWVFGGGTKLTVLGGSDYEFLKSWTVEDLQKRLLALDPMMEQEIEEIRQKYQCKRQPILDAIEAK

SEQ ID NO: 45 - DNA, 519 bp, Artificial Sequence
  VH(112C)-SARAH of 93201 Antibody
atggaggttcagctgcagcagtctggggcagagcttgtgaagccaggggcctcagtcaagttgtcctgcacagcttctggcttcaacattcaagacacctatattcactgggtgaagcagaggcctgaacagggcctggactggattggaaggattgatcctgcgaatggtaatactaaatatgacccgaacttccagggcaaggccactataacagcagacacatcctccaacacagcctacctgcagctcagcagcctggcatctgaggacactgccgtctattactgtgctacctccaattactacagtaggggtgctatggactattggggtcaaggaacctcagtcaccgtctgcagcggatccgactacgagtttcttaagagttggacagtggaggaccttcagaagaggctcttggccctggaccccatgatggagcaggagattgaagagatccggcagaagtaccagtccaagcggcagcccatcctggatgccatagaggctaagtaa

SEQ ID NO: 46 - DNA, 519 bp, Artificial Sequence
  VH(112C)-SARAH of TS2/16 Antibody
atggacgtgaagttggtggagtctgggggaggcttagtgaagcctggagggtccctgaaactctcctgtgcagcctctggattcactttcagtagctataccatgtcttgggttcgccagactccggagaagaggctggagtgggtcgcaaccataagtagtggtggttcttacacctactatccagacagtgtgaagggccgattcaccatttccagagacaaagccaagaacaccctgtatttgcaaatgggcagtctgaagtctgaggacacagccatgtattactgtacaagaataggttacgacgaagattatgctatggaccactggggtcaaggaacctcagtcaccgtctgctcaggatctgactacgagtttcttaagagttggacagtggaggaccttcagaagaggctcttggccctggaccccatgatggagcaggagattgaagagatccggcagaagtaccagtccaagcggcagcccatcctggatgccatagaggctaagtag

SEQ ID NO: 47 - DNA, 513 bp, Artificial Sequence
  VH(112C)-SARAH of SG/19 Antibody
atgcaggttcacctgcagcagtctggagctgagctgatgaagcctggggcctcagtgaagatatcctgcaaggctactggctacacattcactagctactggatagagtgggtaaagcagaggcctggacatggccttgagtggcttggagagattttacctggaagtggttatattcattataatgagaagtttaagggcaaggccacattcactacagatacatcctcaaacacagcctacatgcaactcagcagcctgacatctgaggactctgccgtctattactgttcaagggctctggccctctatgctatggactattggggtcaaggaacctcagtcaccgtctgctcaggatctgactacgagtttcttaagagttggacagtggaggaccttcagaagaggctcttggccctggaccccatgatggagcaggagattgaagagatccggcagaagtaccagtccaagcggcagcccatcctggatgccatagaggctaagtag

SEQ ID NO: 48 - DNA, 525 bp, Artificial Sequence
  VH(112C)-SARAH of t8E4 Antibody
atgaaacaggtgcagctgaaggagtcaggacctgaccttgtgcagccctcacagaccctgtctctcacctgcactgtctctgggttctcattaaccggctatggtgttcactgggttcgccagcctccaggaaagggactggagtgggtgggaacactgggctggaatgacaaaaaatattataattcagctctaaaatctcgactgagcatcagcagggatacctccaagaaccaagttttcttaaaactgagcagtctggaaactgaagacacagccatgtactactgtactagagatggcggcctactattcgcttactatgctatggactactggggtcaaggaacctcagtcaccgtctgcagcggatccgactacgagtttcttaagagttggacagtggaggaccttcagaagaggctcttggccctggaccccatgatggagcaggagattgaagagatccggcagaagtaccagtccaagcggcagcccatcctggatgccatagaggctaagtaa

SEQ ID NO: 49 - DNA, 540 bp, Artificial Sequence
  VH(112C)-SARAH of 9E10 Antibody
atggaagtgaagttggttgaatctgggggagatctggtcaaaccgggagggagcctgaaactgtcatgtgcggcgtctggctttaccttttctcattacgggatgtcctgggtgcggcagactccggataagcgtctggaatgggtcgccaccattgggtcccggggaacctatacacactaccccgactctgtgaaaggccggtttaccatcagtcgcgataacgacaagaatgcactgtatctgcagatgaacagcctgaaatccgaagatacagccatgtattactgcgcgcgccgtagtgagttctactactacggtaacacatactactactcagcaatggactactggggccagggtgctagcgtgactgtttgcagcggatccgactacgagtttcttaagagttggacagtggaggaccttcagaagaggctcttggccctggaccccatgatggagcaggagattgaagagatccggcagaagtaccagtccaagcggcagcccatcctggatgccatagaggctaagtaa

SEQ ID NO: 50 - DNA, 519 bp, Artificial Sequence
  VH(112C)-SARAH of 12CA5 Antibody
atggaagtgaagttggttgaatctgggggagacctggtgaaaccgggcgggagtctgaaactgtcctgtgcggcaagtggctttaccttctcatcctacggcatgtcctgggttcgtcagaccccggataagcgtctggaatgggtcgcaactatttctcggggcggtagttatacctattaccccgattcagtgaaaggccggtttacaatcagccgcgacaacgctaagaatactctgtacctgcagatgagctccctgaaatctgaggataccgccatgtattactgcgcgcgccgtgaaacctatgatgagaaaggtttcgcctactgggggcagggaaccacagtgaccgtttgcagcggatccgactacgagtttcttaagagttggacagtggaggaccttcagaagaggctcttggccctggaccccatgatggagcaggagattgaagagatccggcagaagtaccagtccaagcggcagcccatcctggatgccatagaggctaagtaa

SEQ ID NO: 51 - DNA, 522 bp, Artificial Sequence
  VH(112C)-SARAH of t1E4 Antibody
atgaaacagggtcagctgcagcagtctggacctgagctggtgaagcctggggcctcagtgaagatttcctgcaaggcttctggctatgtcttcagtagctcctggatgaactgggtgaagcagaggcctggaaagggtcttgagtggattggacggatttatcctggatatggagatactaactacaatgggaagttcaagggcaaggccacactgactgcagacaaatcctccagcacagcctacatgcaactcagcagcctgacatctgaggactctgcggtctacttctgtgtaagagaggaactgggaccctactggtacttcgatgtctggggcgcagggaccacggtcaccgtctgcagcggatccgactacgagtttcttaagagttggacagtggaggaccttcagaagaggctcttggccctggaccccatgatggagcaggagattgaagagatccggcagaagtaccagtccaagcggcagcccatcctggatgccatagaggctaagtaa

SEQ ID NO: 52 - DNA, 513 bp, Artificial Sequence
  VH(112C)-SARAH of NZ-1 Antibody
atgaaagaggtgcagctggtggagtctgggggaggcttagtgcagcctggaaggtccctgaaactctcctgtgcagcctcaggattcactttcagtaactatggcatggcctgggtccgccagactccaacgaagggtctggagtggatcgcatccattagtgctggtggtgataaaacttactatggagactccgtgaagggccgattcagtatctccagagataatgcaaaaaccacccactacttgcaaatggacagtctgaggtctgaggacacggccacttattactgtgcaaaaacttcccgggtatattttgattactggggccaaggagtcatggtcacagtctgcagcggatccgactacgagtttcttaagagttggacagtggaggaccttcagaagaggctcttggccctggaccccatgatggagcaggagattgaagagatccggcagaagtaccagtccaagcggcagcccatcctggatgccatagaggctaagtaa

SEQ ID NO: 53 - DNA, 494 bp, Artificial Sequence
  VL-SARAH(37C) of 93201 Antibody
atggacattgtgctcacccaatctccagcttctttggctgtgtctctagggcagagagccaccatctcctgcagagccagtgaaagtgttgaatattatggcacaaatttaatgcactggtaccaacagaaaccaggacagccacccaaactcctcatctatgttgcatccaccgtaaaatctggggtccctgccaggtttagtggcagtgggtctgggacagacttcagcctcaacatccatcctgtggaggaggatgatattgcaatgtatttctgtcagcaaagtaggaaggttccgtggacgttcggtggaggcaccagactggaaatcaaacggggatccgactacgagtttcttaagagttggacagtggaggaccttcagaagaggctcttggccctggaccccatgatggagcaggagattgaagagatccggcagaagtaccagtgcaagcggcagcccatcctggatgccatagaggctaagta

SEQ ID NO: 54 - DNA, 486 bp, Artificial Sequence
  VL-SARAH(37C) of TS2/16 Antibody
atgcagattgttgttacgcagagaccgacaaccatggctgcatctcccggggacaagatcattatcacctgcagtgtcagttcaattataagttccaattacctgcattggtatagtcagaagccaggattctcccctaaactcttgatttataggacatccaatctggcttctggagtcccacctcgcttcagtggcagtgggtctgggacctcttactctctcacaattggcaccatggaggctgaagatgttgccacttactactgccagcagggttctgatattccactcacgttcggtgatgggaccaagctggacctgaaacggggatctgactacgagtttcttaagagttggacagtggaggaccttcagaagaggctcttggccctggaccccatgatggagcaggagattgaagagatccggcagaagtaccagtgcaagcggcagcccatcctggatgccatagaggctaagtag

SEQ ID NO: 55 - DNA, 498 bp, Artificial Sequence
  VL-SARAH(37C) of SG/19 Antibody
atggacatcgttatgactcaggctaccccctctatacctgtcactcctggagagtcagtctccatctcctgcaggtctaataagagtctcctgcatagtaatggcaacacttacttgtattggttcctgcagaggccaggccagtctcctcggctcctgatatttcggatgtccaaccttgcctcaggagtcccagacaggttcagtggcagtgggtcaggaactgctttcacactgagaatcagtagagtggaggctgcggatgtgggtatttatttctgtttgcaacatctagaatatcctttcacgttcggtgctgggaccaagctggagctgaagcggggatctgactacgagtttcttaagagttggacagtggaggaccttcagaagaggctcttggccctggaccccatgatggagcaggagattgaagagatccggcagaagtaccagtgcaagcggcagcccatcctggatgccatagaggctaagtag

SEQ ID NO: 56 - DNA, 483 bp, Artificial Sequence
  VL-SARAH(37C) of t8E4 Antibody
atggatatccagatgacacagactacatcctccctgtctgcctctctgggagacagagtcaccttcagttgcagggcaagtcaggacattagcaattatttaaactggtatcaacagaagccagatggaactgttaaactcctgatcttctacacatcaagattacactcaggagtcccatcaaggttcagtggcagtgggtctgggacagattattctctcactattgccaacctggaacaagaagattttgccacttacttttgccaacaggatagtaagcatccgtttacgttcggatcggggaccaagctggaaataaaacggggatccgactacgagtttcttaagagttggacagtggaggaccttcagaagaggctcttggccctggaccccatgatggagcaggagattgaagagatccggcagaagtaccagtgcaagcggcagcccatcctggatgccatagaggctaagtaa

SEQ ID NO: 57 - DNA, 495 bp, Artificial Sequence
  VL-SARAH(37C) of 9E10 Antibody
atggacatcgttttgactcagtctccggcatccctggcggtctccctggggcagcgggcaactatttcctgtcgggcgagcgaatccgttgataactatgggttttccttcatgaactggtttcagcagaaaccgggccagccgcccaagctgctgatctatgccatcagtaatcgcggatcaggcgtgccagcgcgttttagcggttccgggtctggtactgatttctccctgaacattcacccagtggaagaggatgaccctgccatgtacttttgccagcagaccaaagaagttccgtggaccttcggcggtgggacaaagctggagatcaaagcgggatccgactacgagtttcttaagagttggacagtggaggaccttcagaagaggctcttggccctggaccccatgatggagcaggagattgaagagatccggcagaagtaccagtgcaagcggcagcccatcctggatgccatagaggctaagtaa

SEQ ID NO: 58 - DNA, 501 bp, Artificial Sequence
  VL-SARAH(37C) of 12CA5 Antibody
atggacatcgaattgactcagtctccgtctagcctgaccgttactgcgggagagaaagttacaatgagctgtaagtcttcccagagcctgctgaatagcggcaaccagaaaaactatctgacctggtaccagcagaaacctggtcagccgcccaagctgctgatctattgggcatcaacacgcgaaagcggcgtgcctgatcgttttaccggctctggtagtgggcgggacttcaccctgacaatcagctccgtgcaggccgaagatctggcggtttattactgccagaacgacaattctcacccgctgacttttggagccggcaccaaactggagctgaaagcgggatccgactacgagtttcttaagagttggacagtggaggaccttcagaagaggctcttggccctggaccccatgatggagcaggagattgaagagatccggcagaagtaccagtgcaagcggcagcccatcctggatgccatagaggctaagtaa

SEQ ID NO: 59 - DNA, 498 bp, Artificial Sequence
  VL-SARAH(37C) of t1E4 Antibody
atggatgttgtgatgacccaaactccactctccctgcctgtcagtcttggagatcaagcctccatctcttgcagatctagtcagagccttgtacacagtaatggaaacacctatttacattggtacctgcagaagccaggccagtctccaaagctcctgatctacaaagtttccaaccgattttctggggtcccagacaggttcagtggcagtggatcagggacagatttcacactcaagatcagcagagtggaggctgaggatctgggagtttatttctgctctcaaagtacacatgttccgtatacgttcggatcggggaccaagttggaaataaaacggggatccgactacgagtttcttaagagttggacagtggaggaccttcagaagaggctcttggccctggaccccatgatggagcaggagattgaagagatccggcagaagtaccagtgcaagcggcagcccatcctggatgccatagaggctaagtaa

SEQ ID NO: 60 - DNA, 489 bp, Artificial Sequence
  VL-SARAH(37C) of NZ-1 Antibody
atgcagtttgtgcttactcagccaaactctgtgtctacgaatctcggaagcacagtcaaactgtcttgtaagcgcagcactggtaacattggaagcaattatgtgaactggtaccagcagcatgagggaagatctcccaccactatgatttatagggatgataagagaccagatggagttcctgacaggttctctggctccattgacagatcttccaactcagccctcctgacaatcaataatgtgcagactgaagatgaagctgactacttctgtcactcttacagtagtggtattgttttcggtggtggaaccaagctcactgtcctaggtggatccgactacgagtttcttaagagttggacagtggaggaccttcagaagaggctcttggccctggaccccatgatggagcaggagattgaagagatccggcagaagtaccagtgcaagcggcagcccatcctggatgccatagaggctaagtaa

SEQ ID NO: 61 - protein, 172 aa, Artificial Sequence
  VH(112C)-SARAH of 93201 Antibody
MEVQLQQSGAELVKPGASVKLSCTASGFNIQDTYIHWVKQRPEQGLDWIGRIDPANGNTKYDPNFQGKATITADTSSNTAYLQLSSLASEDTAVYYCATSNYYSRGAMDYWGQGTSVTVCSGSDYEFLKSWTVEDLQKRLLALDPMMEQEIEEIRQKYQSKRQPILDAIEAK

SEQ ID NO: 62 - protein, 172 aa, Artificial Sequence
  VH(112C)-SARAH of TS2/16 Antibody
MDVKLVESGGGLVKPGGSLKLSCAASGFTFSSYTMSWVRQTPEKRLEWVATISSGGSYTYYPDSVKGRFTISRDKAKNTLYLQMGSLKSEDTAMYYCTRIGYDEDYAMDHWGQGTSVTVCSGSDYEFLKSWTVEDLQKRLLALDPMMEQEIEEIRQKYQSKRQPILDAIEAK

SEQ ID NO: 63 - protein, 170 aa, Artificial Sequence
  VH(112C)-SARAH of SG/19 Antibody
MQVHLQQSGAELMKPGASVKISCKATGYTFTSYWIEWVKQRPGHGLEWLGEILPGSGYIHYNEKFKGKATFTTDTSSNTAYMQLSSLTSEDSAVYYCSRALALYAMDYWGQGTSVTVCSGSDYEFLKSWTVEDLQKRLLALDPMMEQEIEEIRQKYQSKRQPILDAIEAK

SEQ ID NO: 64 - protein, 174 aa, Artificial Sequence
  VH(112C)-SARAH of t8E4 Antibody
MKQVQLKESGPDLVQPSQTLSLTCTVSGFSLTGYGVHWVRQPPGKGLEWVGTLGWNDKKYYNSALKSRLSISRDTSKNQVFLKLSSLETEDTAMYYCTRDGGLLFAYYAMDYWGQGTSVTVCSGSDYEFLKSWTVEDLQKRLLALDPMMEQEIEEIRQKYQSKRQPILDAIEAK

SEQ ID NO: 65 - protein, 179 aa, Artificial Sequence
  VH(112C)-SARAH of 9E10 Antibody
MEVKLVESGGDLVKPGGSLKLSCAASGFTFSHYGMSWVRQTPDKRLEWVATIGSRGTYTHYPDSVKGRFTISRDNDKNALYLQMNSLKSEDTAMYYCARRSEFYYYGNTYYYSAMDYWGQGASVTVCSGSDYEFLKSWTVEDLQKRLLALDPMMEQEIEEIRQKYQSKRQPILDAIEAK

SEQ ID NO: 66 - protein, 172 aa, Artificial Sequence
  VH(112C)-SARAH of 12CA5 Antibody
MEVKLVESGGDLVKPGGSLKLSCAASGFTFSSYGMSWVRQTPDKRLEWVATISRGGSYTYYPDSVKGRFTISRDNAKNTLYLQMSSLKSEDTAMYYCARRETYDEKGFAYWGQGTTVTVCSGSDYEFLKSWTVEDLQKRLLALDPMMEQEIEEIRQKYQSKRQPILDAIEAK

SEQ ID NO: 67 - protein, 173 aa, Artificial Sequence
  VH(112C)-SARAH of t1E4 Antibody
MKQGQLQQSGPELVKPGASVKISCKASGYVFSSSWMNWVKQRPGKGLEWIGRIYPGYGDTNYNGKFKGKATLTADKSSSTAYMQLSSLTSEDSAVYFCVREELGPYWYFDVWGAGTTVTVCSGSDYEFLKSWTVEDLQKRLLALDPMMEQEIEEIRQKYQSKRQPILDAIEAK

SEQ ID NO: 68 - protein, 170 aa, Artificial Sequence
  VH(112C)-SARAH of NZ-1 Antibody
MKEVQLVESGGGLVQPGRSLKLSCAASGFTFSNYGMAWVRQTPTKGLEWIASISAGGDKTYYGDSVKGRFSISRDNAKTTHYLQMDSLRSEDTATYYCAKTSRVYFDYWGQGVMVTVCSGSDYEFLKSWTVEDLQKRLLALDPMMEQEIEEIRQKYQSKRQPILDAIEAK

SEQ ID NO: 69 - protein, 164 aa, Artificial Sequence
  VL-SARAH(37C) of 93201 Antibody
MDIVLTQSPASLAVSLGQRATISCRASESVEYYGTNLMHWYQQKPGQPPKLLIYVASTVKSGVPARFSGSGSGTDFSLNIHPVEEDDIAMYFCQQSRKVPWTFGGGTRLEIKRGSDYEFLKSWTVEDLQKRLLALDPMMEQEIEEIRQKYQCKRQPILDAIEAK

SEQ ID NO: 70 - protein, 161 aa, artificial
  VL-SARAH(37C) of TS2/16 Antibody
MQIVVTQRPTTMAASPGDKIIITCSVSSIISSNYLHWYSQKPGFSPKLLIYRTSNLASGVPPRFSGSGSGTSYSLTIGTMEAEDVATYYCQQGSDIPLTFGDGTKLDLKRGSDYEFLKSWTVEDLQKRLLALDPMMEQEIEEIRQKYQCKRQPILDAIEAK

SEQ ID NO: 71 - protein, 165 aa, Artificial Sequence
  VL-SARAH(37C) of SG/19 Antibody
MDIVMTQATPSIPVTPGESVSISCRSNKSLLHSNGNTYLYWFLQRPGQSPRLLIFRMSNLASGVPDRFSGSGSGTAFTLRISRVEAADVGIYFCLQHLEYPFTFGAGTKLELKRGSDYEFLKSWTVEDLQKRLLALDPMMEQEIEEIRQKYQCKRQPILDAIEAK

SEQ ID NO: 72 - protein, 160 aa, Artificial Sequence
  VL-SARAH(37C) of t8E4 Antibody
MDIQMTQTTSSLSASLGDRVTFSCRASQDISNYLNWYQQKPDGTVKLLIFYTSRLHSGVPSRFSGSGSGTDYSLTIANLEQEDFATYFCQQDSKHPFTFGSGTKLEIKRGSDYEFLKSWTVEDLQKRLLALDPMMEQEIEEIRQKYQCKRQPILDAIEAK

SEQ ID NO: 73 - protein, 164 aa, Artificial Sequence
  VL-SARAH(37C) of 9E10 Antibody
MDIVLTQSPASLAVSLGQRATISCRASESVDNYGFSFMNWFQQKPGQPPKLLIYAISNRGSGVPARFSGSGSGTDFSLNIHPVEEDDPAMYFCQQTKEVPWTFGGGTKLEIKAGSDYEFLKSWTVEDLQKRLLALDPMMEQEIEEIRQKYQCKRQPILDAIEAK

SEQ ID NO: 74 - protein, 166 aa, Artificial Sequence
  VL-SARAH(37C) of 12CA5 Antibody
MDIELTQSPSSLTVTAGEKVTMSCKSSQSLLNSGNQKNYLTWYQQKPGQPPKLLIYWASTRESGVPDRFTGSGSGRDFTLTISSVQAEDLAVYYCQNDNSHPLTFGAGTKLELKAGSDYEFLKSWTVEDLQKRLLALDPMMEQEIEEIRQKYQCKRQPILDAIEAK

SEQ ID NO: 75 - protein, 165 aa, Artificial Sequence
  VL-SARAH(37C) of t1E4 Antibody
MDVVMTQTPLSLPVSLGDQASISCRSSQSLVHSNGNTYLHWYLQKPGQSPKLLIYKVSNRFSGVPDRFSGSGSGTDFTLKISRVEAEDLGVYFCSQSTHVPYTFGSGTKLEIKRGSDYEFLKSWTVEDLQKRLLALDPMMEQEIEEIRQKYQCKRQPILDAIEAK

SEQ ID NO: 76 - protein, 162 aa, Artificial Sequence
  VL-SARAH(37C) of NZ-1 Antibody
MQFVLTQPNSVSTNLGSTVKLSCKRSTGNIGSNYVNWYQQHEGRSPTTMIYRDDKRPDGVPDRFSGSIDRSSNSALLTINNVQTEDEADYFCHSYSSGIVFGGGTKLTVLGGSDYEFLKSWTVEDLQKRLLALDPMMEQEIEEIRQKYQCKRQPILDAIEAK

SEQ ID NO: 77 - protein, 677 aa, Artificial Sequence
  SORLA Vps10p Domain
QPEPIKVYGQVSLNDSHNQMVVHWAGEKSNVIVALARDSLALARPKSSDVYVSYDYGKSFKKISDKLNFGLGNRSEAVIAQFYHSPADNKRYIFADAYAQYLWITFDFCNTLQGFSIPFRAADLLLHSKASNLLLGFDRSHPNKQLWKSDDFGQTWIMIQEHVKSFSWGIDPYDKPNTIYIERHEPSGYSTVFRSTDFFQSRENQEVILEEVRDFQLRDKYMFATKVVHLLGSEQQSSVQLWVSFGRKPMRAAQFVTRHPINEYYIADASEDQVFVCVSHSNNRTNLYISEAEGLKFSLSLENVLYYSPGGAGSDTLVRYFANEPFADFHRVEGLQGVYIATLINGSMNEENMRSVITFDKGGTWEFLQAPAFTGYGEKINCELSQGCSLHLAQRLSQLLNLQLRRMPILSKESAPGLIIATGSVGKNLASKTNVYISSSAGARWREALPGPHYYTWGDHGGIITAIAQGMETNELKYSTNEGETWKTFIFSEKPVFVYGLLTEPGEKSTVFTIFGSNKENVHSWLILQVNATDALGVPCTENDYKLWSPSDERGNECLLGHKTVFKRRTPHATCFNGEDFDRPVVVSNCSCTREDYECDFGFKMSEDLSLEVCVPDPEFSGKSYSPPVPCPVGSTYRRTRGYRKISGDTCSGGDVEARLEGELVPCPSRLENLYFQ

SEQ ID NO: 78 - protein, 627 aa, Artificial Sequence
  Integrin  ¿6
FNLDTREDNVIRKYGDPGSLFGFSLAMHWQLQPEDKRLLLVGAPRAEALPLQRANRTGGLYSCDITARGPCTRIEFDNDADPTSESKEDQWMGVTVQSQGPGGKVVTCAHRYEKRQHVNTKQESRDIFGRCYVLSQNLRIEDDMDGGDWSFCDGRLRGHEKFGSCQQGVAATFTKDFHYIVFGAPGTYNWKGIVRVEQKNNTFFDMNIFEDGPYEVGGETEHDESLVPVPANSYLGFSLDSGKGIVSKDEITFVSGAPRANHSGAVVLLKRDMKSAHLLPEHIFDGEGLASSFGYDVAVVDLNKDGWQDIVIGAPQYFDRDGEVGGAVYVYMNQQGRWNNVKPIRLNGTKDSMFGIAVKNIGDINQDGYPDIAVGAPYDDLGKVFIYHGSANGINTKPTQVLKGISPYFGYSIAGNMDLDRNSYPDVAVGSLSDSVTIFRSRPVINIQKTITVTPNRIDLRQKTACGAPSGICLQVKSCFEYTANPAGYNPSISIVGTLEAEKERRKSGLSSRVQFRNQGSEPKYTQELTLKRQKQKVCMEETLWLQDNIRDKLRPIPITASVEIQEPSSRRRVNSLPEVLPILNSDEPKTAHIDVHFLKEGCGDDNVCNSNLKLEYKGSLENLYFQ

SEQ ID NO: 79 - protein, 454 aa, Artificial Sequence
  Integrin  À1
QTDENRCLKANAKSCGECIQAGPNCGWCTNSTFLQEGMPTSARCDDLEALKKKGCPPDDIENPRGSKDIKKNKNVTNRSKGTAEKLKPEDITQIQPQQLVLRLRSGEPQTFTLKFKRAEDYPIDLYYLMDLSYSMKDDLENVKSLGTDLMNEMRRITSDFRIGFGSFVEKTVMPYISTTPAKLRNPCTSEQNCTSPFSYKNVLSLTNKGEVFNELVGKQRISGNLDSPEGGFDAIMQVAVCGSLIGWRNVTRLLVFSTDAGFHFAGDGKLGGIVLPNDGQCHLENNMYTMSHYYDYPSIAHLVQKLSENNIQTIFAVTEEFQPVYKELKNLIPKSAVGTLSANSSNVIQLIIDAYNSLSSEVILENGKLSEGVTISYKSYCKNGVNGTGENGRKCSNISIGDEVQFEISITSNKCPKKDSDSFKIRPLGFTEEVEVILQYICECEGGLENLYFQ

SEQ ID NO: 80 - protein, 350 aa, Artificial Sequence
  HGF
SGQDCYRGNGKNYMGQLSQTRSGLTCSMWDKNMEDLHRHIFWEPDASKLNENYCRNPDDDAHGPWCYTGNPLIPWDYCPISRCEGDTTPGIVNLDHPVISCAKTIEGRVVNGIPTRTNIGWMVSLRYRNKHICGGSLIKESWVLTARQCFPSRDLKDYEAWLGIHDVHGRGDEKCKQVLQVSQLVYGPEGSDLVLMKLARPAVLDDFVSTIDLPNYGCTIPEKTSCSVYGWGYTGLINYDGLLRVAHLYIMGNEKCSQHHRGKVTLQESEICAGAEKIGSGPCEGDYGGPLVCEQHKMRMVLGVIVPGRGCAIPNRPGIFVRVAYYAKWIHKIILTYKVPQSRLENLYFQ

SEQ ID NO: 81 - protein, 197 aa, Artificial Sequence
  T4L Protein
MGEQKLISEEDLRENLYFQGKDGSGHKNIFEMLRIDEGLRLKIYKDTEGYYTIGIGHLLTKSPSLNAAKSELDKAIGRNTNGVITKDEAEKLFNQDVDAAVRGILRNAKLKPVYDSLDAVRRAALINMVFQMGETGVAGFTNSLRMLQQKRWDEAAVNLAKSRWYNQTPNRAKRVITTFRTGTWDAYLEHHHHHHHH

SEQ ID NO: 82 - protein, 196 aa, Artificial Sequence
  T4L Protein
MGYPYDVPDYARENLYFQGKDGSGHKNIFEMLRIDEGLRLKIYKDTEGYYTIGIGHLLTKSPSLNAAKSELDKAIGRNTNGVITKDEAEKLFNQDVDAAVRGILRNAKLKPVYDSLDAVRRAALINMVFQMGETGVAGFTNSLRMLQQKRWDEAAVNLAKSRWYNQTPNRAKRVITTFRTGTWDAYLEHHHHHHHH

SEQ ID NO: 83 - protein, 14 aa, Artificial Sequence
  PA Peptide
EGGVAMPGAEDDVV

SEQ ID NO: 84 - protein, 271 aa, Artificial Sequence
  Sequence for producing scFv of NZ-1 Antibody
MKEVQLVESGGGLVQPGRSLKLSCAASGFTFSNYGMAWVRQTPTKGLEWIASISAGGDKTYYGDSVKGRFSISRDNAKTTHYLQMDSLRSEDTATYYCAKTSRVYFDYWGQGVMVTVSSGGGGSGGGGSGGGGSTQFVLTQPNSVSTNLGSTVKLSCKRSTGNIGSNYVNWYQQHEGRSPTTMIYRDDKRPDGVPDRFSGSIDRSSNSALLTINNVQTEDEADYFCHSYSSGIVFGGGTKLTVLGAAAHHHHHHGAAEQKLISEEDLNGAA

SEQ ID NO: 85 - protein, 170 aa, Artificial Sequence
  VH-SARAH(Y35C) of NZ-1 Antibody
MKEVQLVESGGGLVQPGRSLKLSCAASGFTFSNYGMAWVRQTPTKGLEWIASISAGGDKTYYGDSVKGRFSISRDNAKTTHYLQMDSLRSEDTATYYCAKTSRVYFDYWGQGVMVTVSSGSDYEFLKSWTVEDLQKRLLALDPMMEQEIEEIRQKCQSKRQPILDAIEAK

SEQ ID NO: 86 - protein, 162 aa, Artificial Sequence
  VL-SARAH(M24C) of NZ-1 Antibody
MQFVLTQPNSVSTNLGSTVKLSCKRSTGNIGSNYVNWYQQHEGRSPTTMIYRDDKRPDGVPDRFSGSIDRSSNSALLTINNVQTEDEADYFCHSYSSGIVFGGGTKLTVLGGSDYEFLKSWTVEDLQKRLLALDPMCEQEIEEIRQKYQSKRQPILDAIEAK

SEQ ID NO: 87 - protein, 170 aa, Artificial Sequence
  VH-SARAH(Y35C) of SG/19 Antibody
MQVHLQQSGAELMKPGASVKISCKATGYTFTSYWIEWVKQRPGHGLEWLGEILPGSGYIHYNEKFKGKATFTTDTSSNTAYMQLSSLTSEDSAVYYCSRALALYAMDYWGQGTSVTVSSGSDYEFLKSWTVEDLQKRLLALDPMMEQEIEEIRQKCQSKRQPILDAIEAK

SEQ ID NO: 88 - protein, 166 aa, Artificial Sequence; identical to SEQ ID NO: 29
  VL-SARAH(M24C) of SG/19 Antibody

SEQ ID NO: 89 - protein, 11 aa, Artificial Sequence
  eTEV Peptide
RENLYFQGKDG